European Patent Specification EP 3 845 550 B1, published July 17, 2024. Title: Composition for growth-promoting cell containing erythropoietin-derived peptide. Applicant: Daegu Gyeongbuk Institute of Science and Technology. The sequence listing filed with the application follows.

SEQUENCE LISTING (28 sequences)

SEQ ID NO: 1 - protein, 23 aa, Artificial Sequence
  ML1
LQLHVDKAVSGLRSLTTLLRALG

SEQ ID NO: 2 - protein, 20 aa, Artificial Sequence
  ML2
LHVDKAVSGLRSLTTLLRAL

SEQ ID NO: 3 - protein, 10 aa, Artificial Sequence
  ML3
TKVNFYAWKR

SEQ ID NO: 4 - protein, 24 aa, Artificial Sequence
  ML4
DKAVSGLRSLTTLLRALGAQKEAI

SEQ ID NO: 5 - protein, 14 aa, Artificial Sequence
  ML5
SGLRSLTTLLRALG

SEQ ID NO: 6 - protein, 20 aa, Artificial Sequence
  ML6
SGLRSLTTLLRALGAQKEAI

SEQ ID NO: 7 - protein, 25 aa, Artificial Sequence
  ML7
WEPLQLHVDKAVSGLRSLTTLLRAL

SEQ ID NO: 8 - protein, 17 aa, Artificial Sequence
  ML8
DKAVSGLRSLTTLLRAL

SEQ ID NO: 9 - protein, 23 aa, Artificial Sequence
  ML1-1
LQLHVLKRVSGLLSHTMLLKALG

SEQ ID NO: 10 - protein, 20 aa, Artificial Sequence
  ML2-1
RHVQKAESGLRSLTKLLREL

SEQ ID NO: 11 - protein, 10 aa, Artificial Sequence
  ML3-1
TRVNYQAWKR

SEQ ID NO: 12 - protein, 24 aa, Artificial Sequence
  ML4-1
KKAVSGLKTLTHILRALGAQKEAI

SEQ ID NO: 13 - protein, 14 aa, Artificial Sequence
  ML5-1
AGLRSRAHLRRALA

SEQ ID NO: 14 - protein, 20 aa, Artificial Sequence
  ML6-1
KGLRSLISLLRALGAQKEAI

SEQ ID NO: 15 - protein, 25 aa, Artificial Sequence
  ML7-1
DEALDLEVDKAATGLRTLTTLIRAL

SEQ ID NO: 16 - protein, 13 aa, Artificial Sequence
  ML8-1
NKAVAGLRSLTVN

SEQ ID NO: 17 - protein, 23 aa, Artificial Sequence
  ML1-H1
LQLHVLKAVSGLLTHTTLLKALG

SEQ ID NO: 18 - protein, 23 aa, Artificial Sequence
  ML1-H2
LQLHVLKAVSGLLTLTMIRRALG

SEQ ID NO: 19 - protein, 23 aa, Artificial Sequence
  ML1-H3
LQLHVLKAVAGLRTLAMIRRALA

SEQ ID NO: 20 - protein, 23 aa, Artificial Sequence
  ML1-C1
LDLEVDKAVSGLRSLTTLLRALG

SEQ ID NO: 21 - protein, 23 aa, Artificial Sequence
  ML1-C2
LQRHVDKRVSGLRSLTTLLRALG

SEQ ID NO: 22 - protein, 23 aa, Artificial Sequence
  ML1-C3
LQRHVKKRVKGLKSLTTLLRALG

SEQ ID NO: 23 - protein, 16 aa, Artificial Sequence
  ML1-L2
LHVDKAVSGLRSLTTL

SEQ ID NO: 24 - protein, 16 aa, Artificial Sequence
  ML1-K2
KHVDKAVSGLRSLTTK

SEQ ID NO: 25 - protein, 16 aa, Artificial Sequence
  ML1-R2
RHVDKAVSGLRSLTTR

SEQ ID NO: 26 - protein, 19 aa, Artificial Sequence
  MLP
LHVDKAVSGLRSLTTLLRA

SEQ ID NO: 27 - protein, 19 aa, Artificial Sequence
  MLP-C
RHVKKRVKGLKSLTTLLRA

SEQ ID NO: 28 - protein, 19 aa, Artificial Sequence
  MLP-H
LHVLKAVSGLLTLTMIRRA